European Patent Application EP 4 591 873 A1, published July 30, 2025. Title: 락토바실러스 플란타룸 균주의 병용 요법 및 이를 이용한 암 치료 방법. Applicant: 지아이바이옴. The sequence listing filed with the application follows.

SEQUENCE LISTING (20 sequences)

SEQ ID NO: 1 - DNA, 1424 bp, synthetic construct
  source 1..1424: mol_type = other DNA
tcgaacgaactctggtattgattggtgcttgcatcatgatttacatttgagtgagtggcgaactggtgagtaacacgtgggaaacctgcccagaagcgggggataacacctggaaacagatgctaataccgcataacaacttggaccgcatggtccgagcttgaaagatggcttcggctatcacttttggatggtcccgcggcgtattagctagatggtggggtaacggctcaccatggcaatgatacgtagccgacctgagagggtaatcggccacattgggactgagacacggcccaaactcctacgggaggcagcagtagggaatcttccacaatggacgaaagtctgatggagcaacgccgcgtgagtgaagaagggtttcggctcgtaaaactctgttgttaaagaagaacatatctgagagtaactgttcaggtattgacggtatttaaccagaaagccacggctaactacgtgccagcagccgcggtaatacgtaggtggcaagcgttgtccggatttattgggcgtaaagcgagcgcaggcggttttttaagtctgatgtgaaagccttcggctcaaccgaagaagtgcatcggaaactgggaaacttgagtgcagaagaggacagtggaactccatgtgtagcggtgaaatgcgtagatatatggaagaacaccagtggcgaaggcggctgtctggtctgtaactgacgctgaggctcgaaagtatgggtagcaaacaggattagataccctggtagtccataccgtaaacgatgaatgctaagtgttggagggtttccgcccttcagtgctgcagctaacgcattaagcattccgcctggggagtacggccgcaaggctgaaactcaaaggaattgacgggggcccgcacaagcggtggagcatgtggtttaattcgaagctacgcgaagaaccttaccaggtcttgacatactatgcaaatctaagagattagacgttcccttcggggacatggatacaggtggtgcatggttgtcgtcagctcgtgtcgtgagatgttgggttaagtcccgcaacgagcgcaacccttattatcagttgccagcattaagttgggcactctggtgagactgccggtgacaaaccggaggaaggtggggatgacgtcaaatcatcatgccccttatgacctgggctacacacgtgctacaatggatggtacaacgagttgcgaactcgcgagagtaagctaatctcttaaagccattctcagttcggattgtaggctgcaactcgcctacatgaagtcggaatcgctagtaatcgcggatcagcatgccgcggtgaatacgttcccgggccttgtacacaccgcccgtcacaccatgagagtttgtaacacccaaagtcggtggggtaaccttttaggaacca

SEQ ID NO: 2 - protein, 288 aa, synthetic construct
MGHTRRQGTSPSKCPYLNFFQLLVLAGLSHFCSGVIHVTKEVKEVATLSCGHNVSVEELAQTRIYWQKEKKMVLTMMSGDMNIWPEYKNRTIFDITNNLSIVILALRPSDEGTYECVVLKYEKDAFKREHLAEVTLSVKADFPTPSISDFEIPTSNIRRIICSTSGGFPEPHLSWLENGEELNAINTTVSQDPETELYAVSSKLDFNMTTNHSFMCLIKYGHLRVNQTFNWNTTKQEHFPDNLLPSWAITLISVNGIFVICCLTYCFAPRCRERRRNERLRRESVRPV

SEQ ID NO: 3 - protein, 208 aa, synthetic construct [sequence omitted]

SEQ ID NO: 4 - protein, 133 aa, synthetic construct [sequence omitted]

SEQ ID NO: 5 - protein, 133 aa, synthetic construct
APTSSSTKKTQLQLEHLLLDLQMILNGINNYKNPKLTAMLTAKFYMPKKATELKHLQCLEEELKPLEEVLNLAQSKNFHLRPRDLISNINVIVLELKGSETTFMCEYADETATIVEFLNRWITFCQSIISTLT

SEQ ID NO: 6 - protein, 133 aa, synthetic construct
APTSSSTKKTQLQLEHLLLDLQMILNGINNYKNPKLTAMLTAKFAMPKKATELKHLQCLEEELKPLEEVLNLAQSKNFHLRPRDLISNINVIVLELKGSETTFMCEYADETATIVEFLNRWITFCQSIISTLT

SEQ ID NO: 7 - protein, 133 aa, synthetic construct
APTSSSTKKTQLQLEHLLLDLQMILNGINNYKNPKLTAMLTAKFYMPKKATELKHLQCLERELKPLEEVLNLAQSKNFHLRPRDLISNINVIVLELKGSETTFMCEYADETATIVEFLNRWITFCQSIISTLT

SEQ ID NO: 8 - protein, 133 aa, synthetic construct
APTSSSTKKTQLQLEHLLLDLQMILNGINNYKNPKLTAMLTAKFYMPKKATELKHLQCLEEELKPLEEVLNGAQSKNFHLRPRDLISNINVIVLELKGSETTFMCEYADETATIVEFLNRWITFCQSIISTLT

SEQ ID NO: 9 - protein, 216 aa, synthetic construct
APEAAGGPSVFLFPPKPKDQLMISRTPEVTCVVVDVSQEDPEVQFNWYVDGVEVHNAKTKPREEQFNSTYRVVSVLTVLHQDWLNGKEYKCKVSNKGLPSSIEKTISKAKGQPREPQVYTLPPSQEEMTKNQVSLTCLVKGFYPSDIAVEWESNGQPENNYKTTPPVLDSDGSFFLYSRLTVDKSRWQEGNVFSCSVLHEALHNHYTQKSLSLSLG

SEQ ID NO: 10 - protein, 30 aa, synthetic construct
GSGGGGSGGGGSGGGGSAESKYGPPCPPCP

SEQ ID NO: 11 - protein, 5 aa, synthetic construct
GGGGS

SEQ ID NO: 12 - protein, 592 aa, synthetic construct
VIHVTKEVKEVATLSCGHNVSVEELAQTRIYWQKEKKMVLTMMSGDMNIWPEYKNRTIFDITNNLSIVILALRPSDEGTYECVVLKYEKDAFKREHLAEVTLSVKADFPTPSISDFEIPTSNIRRIICSTSGGFPEPHLSWLENGEELNAINTTVSQDPETELYAVSSKLDFNMTTNHSFMCLIKYGHLRVNQTFNWNTTKQEHFPDNGSGGGGSGGGGSGGGGSAESKYGPPCPPCPAPEAAGGPSVFLFPPKPKDQLMISRTPEVTCVVVDVSQEDPEVQFNWYVDGVEVHNAKTKPREEQFNSTYRVVSVLTVLHQDWLNGKEYKCKVSNKGLPSSIEKTISKAKGQPREPQVYTLPPSQEEMTKNQVSLTCLVKGFYPSDIAVEWESNGQPENNYKTTPPVLDSDGSFFLYSRLTVDKSRWQEGNVFSCSVLHEALHNHYTQKSLSLSLGGGGGSAPTSSSTKKTQLQLEHLLLDLQMILNGINNYKNPKLTAMLTAKFYMPKKATELKHLQCLEEELKPLEEVLNLAQSKNFHLRPRDLISNINVIVLELKGSETTFMCEYADETATIVEFLNRWITFCQSIISTLT

SEQ ID NO: 13 - protein, 592 aa, synthetic construct
VIHVTKEVKEVATLSCGHNVSVEELAQTRIYWQKEKKMVLTMMSGDMNIWPEYKNRTIFDITNNLSIVILALRPSDEGTYECVVLKYEKDAFKREHLAEVTLSVKADFPTPSISDFEIPTSNIRRIICSTSGGFPEPHLSWLENGEELNAINTTVSQDPETELYAVSSKLDFNMTTNHSFMCLIKYGHLRVNQTFNWNTTKQEHFPDNGSGGGGSGGGGSGGGGSAESKYGPPCPPCPAPEAAGGPSVFLFPPKPKDQLMISRTPEVTCVVVDVSQEDPEVQFNWYVDGVEVHNAKTKPREEQFNSTYRVVSVLTVLHQDWLNGKEYKCKVSNKGLPSSIEKTISKAKGQPREPQVYTLPPSQEEMTKNQVSLTCLVKGFYPSDIAVEWESNGQPENNYKTTPPVLDSDGSFFLYSRLTVDKSRWQEGNVFSCSVLHEALHNHYTQKSLSLSLGGGGGSAPTSSSTKKTQLQLEHLLLDLQMILNGINNYKNPKLTAMLTAKFAMPKKATELKHLQCLEEELKPLEEVLNLAQSKNFHLRPRDLISNINVIVLELKGSETTFMCEYADETATIVEFLNRWITFCQSIISTLT

SEQ ID NO: 14 - protein, 592 aa, synthetic construct
VIHVTKEVKEVATLSCGHNVSVEELAQTRIYWQKEKKMVLTMMSGDMNIWPEYKNRTIFDITNNLSIVILALRPSDEGTYECVVLKYEKDAFKREHLAEVTLSVKADFPTPSISDFEIPTSNIRRIICSTSGGFPEPHLSWLENGEELNAINTTVSQDPETELYAVSSKLDFNMTTNHSFMCLIKYGHLRVNQTFNWNTTKQEHFPDNGSGGGGSGGGGSGGGGSAESKYGPPCPPCPAPEAAGGPSVFLFPPKPKDQLMISRTPEVTCVVVDVSQEDPEVQFNWYVDGVEVHNAKTKPREEQFNSTYRVVSVLTVLHQDWLNGKEYKCKVSNKGLPSSIEKTISKAKGQPREPQVYTLPPSQEEMTKNQVSLTCLVKGFYPSDIAVEWESNGQPENNYKTTPPVLDSDGSFFLYSRLTVDKSRWQEGNVFSCSVLHEALHNHYTQKSLSLSLGGGGGSAPTSSSTKKTQLQLEHLLLDLQMILNGINNYKNPKLTAMLTAKFYMPKKATELKHLQCLERELKPLEEVLNLAQSKNFHLRPRDLISNINVIVLELKGSETTFMCEYADETATIVEFLNRWITFCQSIISTLT

SEQ ID NO: 15 - protein, 592 aa, synthetic construct
VIHVTKEVKEVATLSCGHNVSVEELAQTRIYWQKEKKMVLTMMSGDMNIWPEYKNRTIFDITNNLSIVILALRPSDEGTYECVVLKYEKDAFKREHLAEVTLSVKADFPTPSISDFEIPTSNIRRIICSTSGGFPEPHLSWLENGEELNAINTTVSQDPETELYAVSSKLDFNMTTNHSFMCLIKYGHLRVNQTFNWNTTKQEHFPDNGSGGGGSGGGGSGGGGSAESKYGPPCPPCPAPEAAGGPSVFLFPPKPKDQLMISRTPEVTCVVVDVSQEDPEVQFNWYVDGVEVHNAKTKPREEQFNSTYRVVSVLTVLHQDWLNGKEYKCKVSNKGLPSSIEKTISKAKGQPREPQVYTLPPSQEEMTKNQVSLTCLVKGFYPSDIAVEWESNGQPENNYKTTPPVLDSDGSFFLYSRLTVDKSRWQEGNVFSCSVLHEALHNHYTQKSLSLSLGGGGGSAPTSSSTKKTQLQLEHLLLDLQMILNGINNYKNPKLTAMLTAKFYMPKKATELKHLQCLEEELKPLEEVLNGAQSKNFHLRPRDLISNINVIVLELKGSETTFMCEYADETATIVEFLNRWITFCQSIISTLT

SEQ ID NO: 16 - protein, 25 aa, synthetic construct
MDAMLRGLCCVLLLCGAVFVSPSHA

SEQ ID NO: 17 - DNA, 1857 bp, synthetic construct
  source 1..1857: mol_type = other DNA
atggatgctatgctgagaggcctgtgttgcgtgctgctgctgtgtggcgctgtgttcgtgtctccttctcacgctgtgatccacgtgaccaaagaagtgaaagaggtcgccacactgtcctgcggccacaacgtttcagtggaagaactggcccagaccaggatctactggcagaaagaaaagaaaatggtgctgaccatgatgtccggcgacatgaacatctggcctgagtacaagaaccggaccatcttcgacatcaccaacaacctgtccatcgtgattctggccctgaggccttctgatgagggcacctatgagtgcgtggtgctgaagtacgagaaggacgccttcaagcgcgagcacctggctgaagtgacactgtccgtgaaggccgactttcccacaccttccatctccgacttcgagatccctacctccaacatccggcggatcatctgttctacctctggcggctttcctgagcctcacctgtcttggctggaaaacggcgaggaactgaacgccatcaacaccaccgtgtctcaggaccccgaaaccgagctgtacgctgtgtcctccaagctggacttcaacatgaccaccaaccacagcttcatgtgcctgattaagtacggccacctgagagtgaaccagaccttcaactggaacaccaccaagcaagagcacttccctgacaatggatctggcggcggaggttctggcggaggtggaagcggaggcggaggatctgctgagtctaagtatggccctccttgtcctccatgtcctgctccagaagctgctggcggaccctctgtgttcctgtttcctccaaagcctaaggaccagctcatgatctctcggacacccgaagtgacctgcgtggtggtggatgtgtctcaagaggaccctgaggtgcagttcaattggtacgtggacggcgtggaagtgcacaacgccaagaccaagcctagagaggaacagttcaactccacctacagagtggtgtccgtgctgaccgtgctgcaccaggattggctgaacggcaaagagtacaagtgcaaggtgtccaacaagggcctgccttccagcatcgaaaagaccatctccaaggctaagggccagcctagggaaccccaggtttacaccctgcctccaagccaagaggaaatgaccaagaaccaggtgtccctgacctgcctggtcaagggcttctacccttccgacattgccgtggaatgggagtccaatggccagcctgagaacaactacaagaccacacctcctgtgctggactccgacggctccttctttctgtactctcgcctgaccgtggacaagtctagatggcaagagggcaacgtgttctcctgctctgtgctgcacgaggccctgcacaatcactacacccagaagtccctgtctctgtctcttggaggtggtggcggttctgcccctaccagctcctctaccaagaaaacccagctccagttggagcatctgctgctggacctccagatgattctgaacgggatcaacaactataagaaccccaagctgaccgccatgctgaccgctaagttctacatgcccaagaaggccaccgagctgaagcacctccagtgcctggaagaagaactgaagcccctggaagaggtgctgaatctggcccagtccaagaacttccacctgaggccacgggacctgatcagcaacatcaacgtgatcgtgctggaactgaagggctccgagacaacctttatgtgcgagtacgccgacgagacagccaccatcgtggaatttctgaaccggtggatcaccttctgccagagcatcatctccacactgacctgatga

SEQ ID NO: 18 - DNA, 1851 bp, synthetic construct
  source 1..1851: mol_type = other DNA
atggatgctatgctgagaggcctgtgttgcgtgctgctgctgtgtggcgctgtgttcgtgtctccttctcacgctgtgatccacgtgaccaaagaagtgaaagaggtcgccacactgtcctgcggccacaacgtttcagtggaagaactggcccagaccaggatctactggcagaaagaaaagaaaatggtgctgaccatgatgtccggcgacatgaacatctggcctgagtacaagaaccggaccatcttcgacatcaccaacaacctgtccatcgtgattctggccctgaggccttctgatgagggcacctatgagtgcgtggtgctgaagtacgagaaggacgccttcaagcgcgagcacctggctgaagtgacactgtccgtgaaggccgactttcccacaccttccatctccgacttcgagatccctacctccaacatccggcggatcatctgttctacctctggcggctttcctgagcctcacctgtcttggctggaaaacggcgaggaactgaacgccatcaacaccaccgtgtctcaggaccccgaaaccgagctgtacgctgtgtcctccaagctggacttcaacatgaccaccaaccacagcttcatgtgcctgattaagtacggccacctgagagtgaaccagaccttcaactggaacaccaccaagcaagagcacttccctgacaatggatctggcggcggaggttctggcggaggtggaagcggaggcggaggatctgctgagtctaagtatggccctccttgtcctccatgtcctgctccagaagctgctggcggaccctctgtgttcctgtttcctccaaagcctaaggaccagctcatgatctctcggacacccgaagtgacctgcgtggtggtggatgtgtctcaagaggaccctgaggtgcagttcaattggtacgtggacggcgtggaagtgcacaacgccaagaccaagcctagagaggaacagttcaactccacctacagagtggtgtccgtgctgaccgtgctgcaccaggattggctgaacggcaaagagtacaagtgcaaggtgtccaacaagggcctgccttccagcatcgaaaagaccatctccaaggctaagggccagcctagggaaccccaggtttacaccctgcctccaagccaagaggaaatgaccaagaaccaggtgtccctgacctgcctggtcaagggcttctacccttccgacattgccgtggaatgggagtccaatggccagcctgagaacaactacaagaccacacctcctgtgctggactccgacggctccttctttctgtactctcgcctgaccgtggacaagtctagatggcaagagggcaacgtgttctcctgctctgtgctgcacgaggccctgcacaatcactacacccagaagtccctgtctctgtctcttggaggtggtggcggttctgcccctaccagctcctctaccaagaaaacccagctccagttggagcatctgctgctggacctccagatgattctgaacgggatcaacaactataagaaccccaagctgaccgccatgctgaccgctaagttctacatgcccaagaaggccaccgagctgaagcacctccagtgcctggaaagggaactgaagcccctggaagaggtgctgaatctggcccagtccaagaacttccacctgaggccacgggacctgatcagcaacatcaacgtgatcgtgctggaactgaagggctccgagacaacctttatgtgcgagtacgccgacgagacagccaccatcgtggaatttctgaaccggtggatcaccttctgccagagcatcatctccacactgacc

SEQ ID NO: 19 - DNA, 1851 bp, synthetic construct
  source 1..1851: mol_type = other DNA
atggatgctatgctgagaggcctgtgttgcgtgctgctgctgtgtggcgctgtgttcgtgtctccttctcacgctgtgatccacgtgaccaaagaagtgaaagaggtcgccacactgtcctgcggccacaacgtttcagtggaagaactggcccagaccaggatctactggcagaaagaaaagaaaatggtgctgaccatgatgtccggcgacatgaacatctggcctgagtacaagaaccggaccatcttcgacatcaccaacaacctgtccatcgtgattctggccctgaggccttctgatgagggcacctatgagtgcgtggtgctgaagtacgagaaggacgccttcaagcgcgagcacctggctgaagtgacactgtccgtgaaggccgactttcccacaccttccatctccgacttcgagatccctacctccaacatccggcggatcatctgttctacctctggcggctttcctgagcctcacctgtcttggctggaaaacggcgaggaactgaacgccatcaacaccaccgtgtctcaggaccccgaaaccgagctgtacgctgtgtcctccaagctggacttcaacatgaccaccaaccacagcttcatgtgcctgattaagtacggccacctgagagtgaaccagaccttcaactggaacaccaccaagcaagagcacttccctgacaatggatctggcggcggaggttctggcggaggtggaagcggaggcggaggatctgctgagtctaagtatggccctccttgtcctccatgtcctgctccagaagctgctggcggaccctctgtgttcctgtttcctccaaagcctaaggaccagctcatgatctctcggacacccgaagtgacctgcgtggtggtggatgtgtctcaagaggaccctgaggtgcagttcaattggtacgtggacggcgtggaagtgcacaacgccaagaccaagcctagagaggaacagttcaactccacctacagagtggtgtccgtgctgaccgtgctgcaccaggattggctgaacggcaaagagtacaagtgcaaggtgtccaacaagggcctgccttccagcatcgaaaagaccatctccaaggctaagggccagcctagggaaccccaggtttacaccctgcctccaagccaagaggaaatgaccaagaaccaggtgtccctgacctgcctggtcaagggcttctacccttccgacattgccgtggaatgggagtccaatggccagcctgagaacaactacaagaccacacctcctgtgctggactccgacggctccttctttctgtactctcgcctgaccgtggacaagtctagatggcaagagggcaacgtgttctcctgctctgtgctgcacgaggccctgcacaatcactacacccagaagtccctgtctctgtctcttggaggtggtggcggttctgcccctaccagctcctctaccaagaaaacccagctccagttggagcatctgctgctggacctccagatgattctgaacgggatcaacaactataagaaccccaagctgaccgccatgctgaccgctaagttcgccatgcccaagaaggccaccgagctgaagcacctccagtgcctggaagaagaactgaagcccctggaagaggtgctgaatctggcccagtccaagaacttccacctgaggccacgggacctgatcagcaacatcaacgtgatcgtgctggaactgaagggctccgagacaacctttatgtgcgagtacgccgacgagacagccaccatcgtggaatttctgaaccggtggatcaccttctgccagagcatcatctccacactgacc

SEQ ID NO: 20 - DNA, 1857 bp, synthetic construct
  source 1..1857: mol_type = other DNA
atggatgctatgctgagaggcctgtgttgcgtgctgctgctgtgtggcgctgtgttcgtgtctccttctcacgctgtgatccacgtgaccaaagaagtgaaagaggtcgccacactgtcctgcggccacaacgtttcagtggaagaactggcccagaccaggatctactggcagaaagaaaagaaaatggtgctgaccatgatgtccggcgacatgaacatctggcctgagtacaagaaccggaccatcttcgacatcaccaacaacctgtccatcgtgattctggccctgaggccttctgatgagggcacctatgagtgcgtggtgctgaagtacgagaaggacgccttcaagcgcgagcacctggctgaagtgacactgtccgtgaaggccgactttcccacaccttccatctccgacttcgagatccctacctccaacatccggcggatcatctgttctacctctggcggctttcctgagcctcacctgtcttggctggaaaacggcgaggaactgaacgccatcaacaccaccgtgtctcaggaccccgaaaccgagctgtacgctgtgtcctccaagctggacttcaacatgaccaccaaccacagcttcatgtgcctgattaagtacggccacctgagagtgaaccagaccttcaactggaacaccaccaagcaagagcacttccctgacaatggatctggcggcggaggttctggcggaggtggaagcggaggcggaggatctgctgagtctaagtatggccctccttgtcctccatgtcctgctccagaagctgctggcggaccctctgtgttcctgtttcctccaaagcctaaggaccagctcatgatctctcggacacccgaagtgacctgcgtggtggtggatgtgtctcaagaggaccctgaggtgcagttcaattggtacgtggacggcgtggaagtgcacaacgccaagaccaagcctagagaggaacagttcaactccacctacagagtggtgtccgtgctgaccgtgctgcaccaggattggctgaacggcaaagagtacaagtgcaaggtgtccaacaagggcctgccttccagcatcgaaaagaccatctccaaggctaagggccagcctagggaaccccaggtttacaccctgcctccaagccaagaggaaatgaccaagaaccaggtgtccctgacctgcctggtcaagggcttctacccttccgacattgccgtggaatgggagtccaatggccagcctgagaacaactacaagaccacacctcctgtgctggactccgacggctccttctttctgtactctcgcctgaccgtggacaagtctagatggcaagagggcaacgtgttctcctgctctgtgctgcacgaggccctgcacaatcactacacccagaagtccctgtctctgtctcttggaggtggtggcggttctgcccctaccagctcctctaccaagaaaacccagctccagttggagcatctgctgctggacctccagatgattctgaacgggatcaacaactataagaaccccaagctgaccgccatgctgaccgctaagttctacatgcccaagaaggccaccgagctgaagcacctccagtgcctggaagaagaactgaagcccctggaagaggtgctgaatggggcccagtccaagaacttccacctgaggccacgggacctgatcagcaacatcaacgtgatcgtgctggaactgaagggctccgagacaacctttatgtgcgagtacgccgacgagacagccaccatcgtggaatttctgaaccggtggatcaccttctgccagagcatcatctccacactgacctgatga